European Patent Application EP 4 257 689 A1, published October 11, 2023. Title: Novel promoter variant for constitutive expression and use of the same. Applicant: DAESANG CORPORATION. The sequence listing filed with the application follows.

SEQUENCE LISTING (10 sequences)

SEQ ID NO: 1 - DNA, 137 bp, Unknown
  Promoter gapA
aggcgagtcagtcgcgtaatgcttaggcacaggattgatttgtcgcaatgattgacacgattccgcttgacgctgcgtaaggtttttgtaattttacaggcaaccttttattcactaacaaatagctggaggaatat

SEQ ID NO: 2 - DNA, 115 bp, Unknown
  Promoter BLMA
ggtgtctcattctgttaccgttaacagctgaaaatgattgttcctgttaccgccgtcatgataatttcagaataaaagccggtttatcacagccggacaaccaaaagggggaaac

SEQ ID NO: 3 - protein, 294 aa, Unknown
  Wild type D-allulose 3-epimerase derived from Flavonifractor plautii
MNPIGMHYGFWSHNWDEIAYIPLMEKLAWLGFDICEVASAEWGYYDDARLRELKACADHNGLGITYSIGLEAKYDLASDDPAVRENGIRHVTRILESMPKVGAAILNGVSYAGWQALPDHGITLDEKRRKEELALESMSRLMKVAEDCGVLYCCEVVNRFEQYLLNTAKEGVEFVKRLGSPNARVLLDTFHMNIEEDSMVDAILEAGPWLGHFHVGENNRRPAGSTNRLPWKDMAAALKQVNYQGAIVMEPFVLMGGTIPYDIKVWRDLSGGAGEAGLDEMAGRACRFLKELTA

SEQ ID NO: 4 - DNA, 885 bp, Unknown
  Polynucleotide coding wild type D-allulose 3-epimerase derived from Flavonifractor plautii
atgaacccgattggaatgcactacggcttctggagccacaactgggacgagattgcatacatacccctgatggagaagctggcctggctgggctttgacatctgcgaggtggcctccgccgagtggggctattacgacgacgccaggctgcgggagctgaaggcctgcgccgatcacaacggcctgggcatcacctattccatcggcctggaggccaaatacgacctggccagcgacgatccggcggtgcgggagaacggcatccgccatgtcacccgcatcctggagagcatgcccaaggtgggggcggccatcctcaacggcgtgtcctacgccgggtggcaggccctgcccgaccacggaatcaccctggacgagaagcgccgcaaggaggagcttgccctggagtccatgtcccggctcatgaaggtggcggaggactgcggcgtgctctactgctgcgaggtggtcaaccgcttcgagcagtacctgctcaacaccgccaaagagggcgtggagtttgtcaagcgcctgggcagtcccaacgcccgggtgctgctggataccttccacatgaacatcgaggaggacagcatggtggacgccattctggaggcgggcccctggctggggcatttccacgtgggggagaacaaccgccgccccgccggctccaccaaccgcctgccctggaaggacatggccgccgccctcaagcaggtgaactaccagggggccattgtgatggagcccttcgtgctcatggggggtaccattccctatgatatcaaggtctggcgggatctcagcggcggggccggggaggccgggctggacgagatggcgggccgggcctgccggttcctcaaggagctgaccgcgtaa

SEQ ID NO: 5 - protein, 294 aa, Artificial Sequence
  D-allulose 3-epimerase variant W29K/G216S/M234I
MNPIGMHYGFWSHNWDEIAYIPLMEKLAKLGFDICEVASAEWGYYDDARLRELKACADHNGLGITYSIGLEAKYDLASDDPAVRENGIRHVTRILESMPKVGAAILNGVSYAGWQALPDHGITLDEKRRKEELALESMSRLMKVAEDCGVLYCCEVVNRFEQYLLNTAKEGVEFVKRLGSPNARVLLDTFHMNIEEDSMVDAILEAGPWLGHFHVSENNRRPAGSTNRLPWKDIAAALKQVNYQGAIVMEPFVLMGGTIPYDIKVWRDLSGGAGEAGLDEMAGRACRFLKELTA

SEQ ID NO: 6 - DNA, 885 bp, Artificial Sequence
  Polynucleotide coding D-allulose 3-epimerase variant W29K/G216S/M234I
atgaacccgattggaatgcactacggcttctggagccacaactgggacgagattgcatacatacccctgatggagaagctggccaaactgggctttgacatctgcgaggtggcctccgccgagtggggctattacgacgacgccaggctgcgggagctgaaggcctgcgccgatcacaacggcctgggcatcacctattccatcggcctggaggccaaatacgacctggccagcgacgatccggcggtgcgggagaacggcatccgccatgtcacccgcatcctggagagcatgcccaaggtgggggcggccatcctcaacggcgtgtcctacgccgggtggcaggccctgcccgaccacggaatcaccctggacgagaagcgccgcaaggaggagcttgccctggagtccatgtcccggctcatgaaggtggcggaggactgcggcgtgctctactgctgcgaggtggtcaaccgcttcgagcagtacctgctcaacaccgccaaagagggcgtggagtttgtcaagcgcctgggcagtcccaacgcccgggtgctgctggataccttccacatgaacatcgaggaggacagcatggtggacgccattctggaggcgggcccctggctggggcatttccacgtgagcgagaacaaccgccgccccgccggctccaccaaccgcctgccctggaaggacattgccgccgccctcaagcaggtgaactaccagggggccattgtgatggagcccttcgtgctcatggggggtaccattccctatgatatcaaggtctggcgggatctcagcggcggggccggggaggccgggctggacgagatggcgggccgggcctgccggttcctcaaggagctgaccgcgtaa

SEQ ID NO: 7 - protein, 294 aa, Artificial Sequence
  D-allulose 3-epimerase variant W29K/A77S/G216S/M234I
MNPIGMHYGFWSHNWDEIAYIPLMEKLAKLGFDICEVASAEWGYYDDARLRELKACADHNGLGITYSIGLEAKYDLSSDDPAVRENGIRHVTRILESMPKVGAAILNGVSYAGWQALPDHGITLDEKRRKEELALESMSRLMKVAEDCGVLYCCEVVNRFEQYLLNTAKEGVEFVKRLGSPNARVLLDTFHMNIEEDSMVDAILEAGPWLGHFHVSENNRRPAGSTNRLPWKDIAAALKQVNYQGAIVMEPFVLMGGTIPYDIKVWRDLSGGAGEAGLDEMAGRACRFLKELTA

SEQ ID NO: 8 - DNA, 885 bp, Artificial Sequence
  Polynucleotide coding D-allulose 3-epimerase variant W29K/A77S/G216S/M234I
atgaacccgattggaatgcactacggcttctggagccacaactgggacgagattgcatacatacccctgatggagaagctggccaaactgggctttgacatctgcgaggtggcctccgccgagtggggctattacgacgacgccaggctgcgggagctgaaggcctgcgccgatcacaacggcctgggcatcacctattccatcggcctggaggccaaatacgacctgagcagcgacgatccggcggtgcgggagaacggcatccgccatgtcacccgcatcctggagagcatgcccaaggtgggggcggccatcctcaacggcgtgtcctacgccgggtggcaggccctgcccgaccacggaatcaccctggacgagaagcgccgcaaggaggagcttgccctggagtccatgtcccggctcatgaaggtggcggaggactgcggcgtgctctactgctgcgaggtggtcaaccgcttcgagcagtacctgctcaacaccgccaaagagggcgtggagtttgtcaagcgcctgggcagtcccaacgcccgggtgctgctggataccttccacatgaacatcgaggaggacagcatggtggacgccattctggaggcgggcccctggctggggcatttccacgtgagcgagaacaaccgccgccccgccggctccaccaaccgcctgccctggaaggacattgccgccgccctcaagcaggtgaactaccagggggccattgtgatggagcccttcgtgctcatggggggtaccattccctatgatatcaaggtctggcgggatctcagcggcggggccggggaggccgggctggacgagatggcgggccgggcctgccggttcctcaaggagctgaccgcgtaa

SEQ ID NO: 9 - DNA, 136 bp, Artificial Sequence
  Promoter gapAm1
aggcgagtcagtcgcgtaatgcttaggcacaggattgatttgtcgcaatgattgacacgattccgcttgacgctgcgtaaggtttttgtaattttacaggcaaccttttattcactaacaaatagctggggaatat

SEQ ID NO: 10 - DNA, 132 bp, Artificial Sequence
  Promoter gapAm2
aggcgagtcagtcgcgtaatgcttaggcacaggattgatttgtcgcaatgattgacacgattccgcttgacgctgcgtaaggtttttgtaattttacaggcaaccttttattcactaacaaatagctggagt